European Patent Specification EP 3 665 286 B1, published September 13, 2023. Title: CELL-FREE PROTEIN EXPRESSION USING DOUBLE-STRANDED CONCATAMERIC DNA. Applicant: KVAM, ERIK LEEMING NELSON, JOHN RICHARD GAO, WEI. The sequence listing filed with the application follows.

SEQUENCE LISTING (9 sequences)

SEQ ID NO: 1 - protein, 21 aa, Artificial Sequence
  Description of Artificial Sequence: Synthetic peptide
  MOD_RES (1)..(3): May or may not be present
GSGEGRGSLLTCGDVEENPGP

SEQ ID NO: 2 - protein, 22 aa, Artificial Sequence
  Description of Artificial Sequence: Synthetic peptide
  MOD_RES (1)..(3): May or may not be present
GSGATNFSLLKQAGDVEENPGP

SEQ ID NO: 3 - protein, 23 aa, Artificial Sequence
  Description of Artificial Sequence: Synthetic peptide
  MOD_RES (1)..(3): May or may not be present
GSGQCTNYALLKLAGDVESNPGP

SEQ ID NO: 4 - protein, 25 aa, Artificial Sequence
  Description of Artificial Sequence: Synthetic peptide
  MOD_RES (1)..(3): May or may not be present
GSGVKQTLNFDLLKLAGDVESNPGP

SEQ ID NO: 5 - DNA, 1395 bp, Artificial Sequence
  Description of Artificial Sequence: Synthetic polynucleotide
ccgggatcccagtgaattgtaatacgactcactatagggcgaattaattccggttattttccaccatattgccgtcttttggcaatgtgagggcccggaaacctggccctgtcttcttgacgagcattcctaggggtctttcccctctcgccaaaggaatgcaaggtctgttgaatgtcgtgaaggaagcagttcctctggaagcttcttgaagacaaacaacgtctgtagcgaccctttgcaggcagcggaaccccccacctggcgacaggtgcctctgcggccaaaagccacgtgtataagatacacctgcaaaggcggcacaaccccagtgccacgttgtgagttggatagttgtggaaagagtcaaatggctcacctcaagcgtattcaacaaggggctgaaggatgcccagaaggtaccccattgtatgggatctgatctggggcctcggtgcacatgctttacatgtgtttagtcgaggttaaaaaacgtctaggccccccgaaccacggggacgtggttttcctttgaaaaacacgatgataatatggccacaaccgtgagcaagggcgaggagctgttcaccggggtggtgcccatcctggtcgagctggacggcgacgtaaacggccacaagttcagcgtgtccggcgagggtgaaggcgacgctacttacggaaagctgacactgaagttcatttgcaccacaggcaaactgcctgtgccctggccaaccctcgtgactaccctcacatacggcgtgcagtgctttagcagatatcctgatcatatgaaacagcacgacttctttaagtctgctatgcctgaaggatacgtgcaggagagaaccatcttcttcaaggacgacggaaactataagactagagccgaggtgaagtttgagggagacacactggtgaataggatcgagctgaagggcattgacttcaaggaggacggaaacatcctgggccacaagctggagtacaactacaatagccacaacgtctatattatggctgataagcagaagaacggaatcaaggtgaacttcaagatcagacacaacatcgaggacggcagcgtgcagctggccgaccactaccagcagaatacccctatcggagacggccccgtgctcctgccagacaaccactacctgagcacccagtccgccctgagcaaagaccccaacgagaagcgcgatcatatggttctgctggagttcgtgaccgccgccggcatcactcttggtatggacgagctgtacaagtaataagatctgactgaaaaaaaaaaagtttaaacactagtccgctgagcaataactagcataaccccttggggcctctaaacgggtcttgaggggttttttgctgcagagatctccg

SEQ ID NO: 6 - DNA, 6 bp, Artificial Sequence
  Description of Artificial Sequence: Synthetic oligonucleotide
  Description of Combined DNA/RNA Molecule: Synthetic oligonucleotide
  modified_base (1)..(2): A, C, G, or T/U
  modified_base (1)..(2): Locked nucleic acid
  modified_base (3)..(5): 2-amino dA, 2-thio dT, normal G or normal C
  misc_feature (5)..(6): Phosphorothioate linkage between nucleotides
  modified_base (6)..(6): A, C, G, or T/U
nnnnnn

SEQ ID NO: 7 - DNA, 6 bp, Artificial Sequence
  Description of Artificial Sequence: Synthetic oligonucleotide
  Description of Combined DNA/RNA Molecule: Synthetic oligonucleotide
  5'-biotin
  modified_base (1)..(6): A, C, G, or T/U
  misc_feature (4)..(6): Phosphorothioate linkage between nucleotides
nnnnnn

SEQ ID NO: 8 - protein, 6 aa, Artificial Sequence
  Description of Artificial Sequence: Synthetic 6xHis tag
HHHHHH

SEQ ID NO: 9 - protein, 8 aa, Artificial Sequence
  Description of Artificial Sequence: Synthetic peptide
DYKDDDDK